European Patent Application EP 4 595 967 A1, published August 6, 2025. Title: BACILLUS STRAIN EXPRESSING SUPEROXIDE DISMUTASE, BACILLUS STRAIN SPORES AND/OR SUPEROXIDE DISMUTASE, AND USES THEREOF FOR PREVENTING OR TREATING OF FIBROTIC DISEASES. Applicant: GENOFOCUS, INC. Application KR. The sequence listing filed with the application follows.

SEQUENCE LISTING (59 sequences)

SEQ ID NO: 1 - DNA, 606 bp, Bacillus velezensis
  source 1..606: mol_type = other DNA; note = Nucleotide sequence of SodA
atggcttacaaacttccagaattgccttacgcttatgatgctttagaacctcatatcgataaggaaacgatgacgattcaccatacgaagcaccataacacatacgtgacaaacctcaacaaagcgatcgaaggatctgcgcttgcagagaaatctgtagatgagcttgttgctgatttgaacgcagtgccggaggacatccgcacggcagtccgcaacaatggcggcggacatgcaaaccactctttattctggactcttttatctccgaacggcggaggcgaaccgactggtgagcttgctgaagagatcaaaagcacgttcggaagcttcgatcaatttaaagaaaaattcgccgcagcagctgcaggccgtttcggttcaggctgggcttggctcgttgtaaacaacggcaaacttgaaattacaagcacgccaaaccaagattcaccgctttcagaaggtaaaacacctgttctcggtcttgatgtttgggagcatgcgtactacctgaactaccaaaaccgccgtcctgattacatttcagctttctggaatgttgtgaactgggatgaagttgcccgtctttacagcgaagcaaaataa

SEQ ID NO: 2 - protein, 201 aa, Bacillus velezensis
  source 1..201: note = Amino acid sequence of SodA
MAYKLPELPYAYDALEPHIDKETMTIHHTKHHNTYVTNLNKAIEGSALAEKSVDELVADLNAVPEDIRTAVRNNGGGHANHSLFWTLLSPNGGGEPTGELAEEIKSTFGSFDQFKEKFAAAAAGRFGSGWAWLVVNNGKLEITSTPNQDSPLSEGKTPVLGLDVWEHAYYLNYQNRRPDYISAFWNVVNWDEVARLYSEAK

SEQ ID NO: 3 - DNA, 606 bp, Bacillus velezensis
  source 1..606: mol_type = other DNA; note = Nucleotide sequence of SodA2
atggcttacaaacttccagaattgccttacgcttatgatgctttagaacctcatatcgataaggaaacgatgacgattcaccatacgaagcaccataacacatacgtgacaaacctcaacaaagcgatcgaaggatctgcgcttgcagagaaatctgtagatgagcttgttgctgatttgaacgcagtgccggaggacatccgcacggcagtccgcaacgatggcggcggacatgcaaaccactctttattctggactcttttatctccgaacggcggaggcgaaccgactggtgagcttgctgaagagatcaaaagcacgttcggaagcttcgatcaatttaaagaaaaattcgccgcagcagctgcaggccgtttcggttcaggctgggcttggctcgttgtaaacgacggcaaacttgaaattacaagcacgccaaaccaagattcaccgctttcagaaggtaaaacacctgttctcggtcttgatgtttgggagcatgcgtactacctgaactaccaaaaccgccgtcctgattacatttcagctttctggaatgttgtgaactgggatgaagttgcccgtctttacagcgaagcaaaataa

SEQ ID NO: 4 - protein, 201 aa, Bacillus velezensis
  source 1..201: note = Amino acid sequence of SodA2
MAYKLPELPYAYDALEPHIDKETMTIHHTKHHNTYVTNLNKAIEGSALAEKSVDELVADLNAVPEDIRTAVRNDGGGHANHSLFWTLLSPNGGGEPTGELAEEIKSTFGSFDQFKEKFAAAAAGRFGSGWAWLVVNDGKLEITSTPNQDSPLSEGKTPVLGLDVWEHAYYLNYQNRRPDYISAFWNVVNWDEVARLYSEAK

SEQ ID NO: 5 - protein, 200 aa, Bacillus velezensis
  source 1..200: note = Amino acid sequence of Met-deleted SodA
AYKLPELPYAYDALEPHIDKETMTIHHTKHHNTYVTNLNKAIEGSALAEKSVDELVADLNAVPEDIRTAVRNNGGGHANHSLFWTLLSPNGGGEPTGELAEEIKSTFGSFDQFKEKFAAAAAGRFGSGWAWLVVNNGKLEITSTPNQDSPLSEGKTPVLGLDVWEHAYYLNYQNRRPDYISAFWNVVNWDEVARLYSEAK

SEQ ID NO: 6 - protein, 200 aa, Bacillus velezensis
  source 1..200: note = Amino acid sequence of Met-deleted SodA2
AYKLPELPYAYDALEPHIDKETMTIHHTKHHNTYVTNLNKAIEGSALAEKSVDELVADLNAVPEDIRTAVRNDGGGHANHSLFWTLLSPNGGGEPTGELAEEIKSTFGSFDQFKEKFAAAAAGRFGSGWAWLVVNDGKLEITSTPNQDSPLSEGKTPVLGLDVWEHAYYLNYQNRRPDYISAFWNVVNWDEVARLYSEAK

SEQ ID NO: 7 - DNA, 29 bp, Bacillus velezensis
  source 1..29: mol_type = other DNA; note = Promoter of GF423
ttgattaccacgctttcttttgttacatt

SEQ ID NO: 8 - DNA, 30 bp, Bacillus velezensis
  source 1..30: mol_type = other DNA; note = Promoter of GF427
ttgactttacgctttcttataggttataat

SEQ ID NO: 9 - DNA, 34 bp, unidentified
  source 1..34: mol_type = other DNA; note = SOD up F (Primer)
tccagatcctctacgggcgctgcgtatgctggaa

SEQ ID NO: 10 - DNA, 34 bp, unidentified
  source 1..34: mol_type = other DNA; note = Psodmut R (Primer)
aacttttctaatctcattataacaaaagaaagcg

SEQ ID NO: 11 - DNA, 34 bp, unidentified
  source 1..34: mol_type = other DNA; note = Psodmut F (Primer)
cgctttcttttgttataatgagattagaaaagtt

SEQ ID NO: 12 - DNA, 34 bp, unidentified
  source 1..34: mol_type = other DNA; note = SOD dw R (Primer)
gagttttcgttcggatctgtcctccggcactgcg

SEQ ID NO: 13 - DNA, 32 bp, unidentified
  source 1..32: mol_type = other DNA; note = SOD PF (Primer)
gtaatggaataagccgaaagcttccagagctg

SEQ ID NO: 14 - DNA, 48 bp, unidentified
  source 1..48: mol_type = other DNA; note = SOD P3R (Primer)
attataacctataagaaagcgtaaagtcaatgaaaaagctcacaatcc

SEQ ID NO: 15 - DNA, 46 bp, unidentified
  source 1..46: mol_type = other DNA; note = SOD P3F (Primer)
ttgactttacgctttcttataggttataatgagattagaaaagttc

SEQ ID NO: 16 - DNA, 32 bp, unidentified
  source 1..32: mol_type = other DNA; note = SOD PR (Primer)
catcgtttccttatcgatatgaggttctaaag

SEQ ID NO: 17 - DNA, 23 bp, unidentified
  source 1..23: mol_type = other DNA; note = Cm C F (Primer)
ccgctatctttacaggtacatca

SEQ ID NO: 18 - DNA, 19 bp, unidentified
  source 1..19: mol_type = other DNA; note = SOD mid R (Primer)
gaaccgaaacggcctgcag

SEQ ID NO: 19 - DNA, 20 bp, unidentified
  source 1..20: mol_type = other DNA; note = 424 conf F (Primer)
ggcaggcattatattaggcc

SEQ ID NO: 20 - DNA, 20 bp, unidentified
  source 1..20: mol_type = other DNA; note = 424 conf R (Primer)
gcactgcgttcaaatcagca

SEQ ID NO: 21 - DNA, 20 bp, unidentified
  source 1..20: mol_type = other DNA; note = SOD DC F2 (Primer)
ggattcagcgcttcaaaatc

SEQ ID NO: 22 - DNA, 23 bp, unidentified
  source 1..23: mol_type = other DNA; note = -10 SOD R (Primer)
cgcgaacttttctaatctcatta

SEQ ID NO: 23 - DNA, 20 bp, unidentified
  source 1..20: mol_type = other DNA; note = SOD P2-R (Primer)
ctaatctcattataacctat

SEQ ID NO: 24 - DNA, 34 bp, unidentified
  source 1..34: mol_type = other DNA; note = cm conf F (Primer)
acctttctgatgtagagaaatataatggttcggg

SEQ ID NO: 25 - DNA, 33 bp, unidentified
  source 1..33: mol_type = other DNA; note = cm conf R (Primer)
cggcattatctcatattataaaagccagtcatt

SEQ ID NO: 26 - DNA, 19 bp, unidentified
  source 1..19: mol_type = other DNA; note = Col1a1 (Primer F)
gctcctcttaggggccact

SEQ ID NO: 27 - DNA, 19 bp, unidentified
  source 1..19: mol_type = other DNA; note = Col1a1 (Primer R)
ccacgtctcaccattgggg

SEQ ID NO: 28 - DNA, 19 bp, unidentified
  source 1..19: mol_type = other DNA; note = alpha-SMA (Primer F)
gctcctcttaggggccact

SEQ ID NO: 29 - DNA, 21 bp, unidentified
  source 1..21: mol_type = other DNA; note = alpha-SMA (Primer R)
cccagacatcagggagtaatg

SEQ ID NO: 30 - DNA, 21 bp, unidentified
  source 1..21: mol_type = other DNA; note = TGF-beta1 (Primer F)
agaccacatcagcattgagtg

SEQ ID NO: 31 - DNA, 21 bp, unidentified
  source 1..21: mol_type = other DNA; note = TGF-beta1 (Primer R)
ggtggcaacgaatgtagctgt

SEQ ID NO: 32 - DNA, 19 bp, unidentified
  source 1..19: mol_type = other DNA; note = CTGF (Primer F)
gggcctcttctgcgatttc

SEQ ID NO: 33 - DNA, 21 bp, unidentified
  source 1..21: mol_type = other DNA; note = CTGF (Primer R)
atccaggcaagtgcattggta

SEQ ID NO: 34 - DNA, 21 bp, unidentified
  source 1..21: mol_type = other DNA; note = IL-6 (Primer F)
caaagccagagtccttcagag

SEQ ID NO: 35 - DNA, 20 bp, unidentified
  source 1..20: mol_type = other DNA; note = IL-6 (Primer R)
gtccttagccactccttctg

SEQ ID NO: 36 - DNA, 22 bp, unidentified
  source 1..22: mol_type = other DNA; note = TNF-alpha (Primer F)
cttctgtctactgaacttcggg

SEQ ID NO: 37 - DNA, 22 bp, unidentified
  source 1..22: mol_type = other DNA; note = TNF-alpha (Primer R)
caggcttgtcactcgaattttg

SEQ ID NO: 38 - DNA, 20 bp, unidentified
  source 1..20: mol_type = other DNA; note = IL-1beta (Primer F)
acggaccccaaaagatgaag

SEQ ID NO: 39 - DNA, 20 bp, unidentified
  source 1..20: mol_type = other DNA; note = IL-1beta (Primer R)
ttctccacagccacaatgag

SEQ ID NO: 40 - DNA, 20 bp, unidentified
  source 1..20: mol_type = other DNA; note = 18S rRNA (Primer F)
cagcgtggtcaggatagaac

SEQ ID NO: 41 - DNA, 21 bp, unidentified
  source 1..21: mol_type = other DNA; note = 18S rRNA (Primer R)
cttgatttgaatgcagcggac

SEQ ID NO: 42 - DNA, 28 bp, unidentified
  source 1..28: mol_type = other DNA; note = sodA upstream fragment (Primer #1)
aaacagctgggatgaacacaagtgagag

SEQ ID NO: 43 - DNA, 40 bp, unidentified
  source 1..40: mol_type = other DNA; note = sodA upstream fragment (Primer #2)
cacactcttaagtttgcttccaattctggaagtttgtaag

SEQ ID NO: 44 - DNA, 40 bp, unidentified
  source 1..40: mol_type = other DNA; note = sodA downstream fragment (Primer #1)
ctactgacagcttccaaggatacctgaactaccaaaaccg

SEQ ID NO: 45 - DNA, 29 bp, unidentified
  source 1..29: mol_type = other DNA; note = sodA downstream fragment (Primer #2)
aaacagctgaagctcatgaccacagcaag

SEQ ID NO: 46 - DNA, 20 bp, unidentified
  source 1..20: mol_type = other DNA; note = EmR (Primer #1)
gaagcaaacttaagagtgtg

SEQ ID NO: 47 - DNA, 20 bp, unidentified
  source 1..20: mol_type = other DNA; note = EmR (Primer #2)
tccttggaagctgtcagtag

SEQ ID NO: 48 - DNA, 22 bp, unidentified
  source 1..22: mol_type = other DNA; note = SP-D (Primer F)
aggtccagttggacccaaagga

SEQ ID NO: 49 - DNA, 23 bp, unidentified
  source 1..23: mol_type = other DNA; note = SP-D (Primer R)
ctggtttgccttgaggtcctatg

SEQ ID NO: 50 - DNA, 22 bp, unidentified
  source 1..22: mol_type = other DNA; note = MMP-7 (Primer F)
aggtgtggagtgccagatgttg

SEQ ID NO: 51 - DNA, 22 bp, unidentified
  source 1..22: mol_type = other DNA; note = MMP-7 (Primer R)
ccactacgatccgaggtaagtc

SEQ ID NO: 52 - DNA, 22 bp, unidentified
  source 1..22: mol_type = other DNA; note = tenascin-C (Primer F)
gagacctgacacggagtatgag

SEQ ID NO: 53 - DNA, 23 bp, unidentified
  source 1..23: mol_type = other DNA; note = tenascin-C (Primer R)
ctccaaggtgatgctgttgtctg

SEQ ID NO: 54 - DNA, 22 bp, unidentified
  source 1..22: mol_type = other DNA; note = periostin (Primer F)
cagcaaaccactttcaccgacc

SEQ ID NO: 55 - DNA, 22 bp, unidentified
  source 1..22: mol_type = other DNA; note = periostin (Primer R)
agaaggcgttggtccatgctca

SEQ ID NO: 56 - DNA, 24 bp, unidentified
  source 1..24: mol_type = other DNA; note = CXCK13 (Primer F)
catagatcggattcaagttacgcc

SEQ ID NO: 57 - DNA, 23 bp, unidentified
  source 1..23: mol_type = other DNA; note = CXCK13 (Primer R)
gtaaccatttggcacgaggattc

SEQ ID NO: 58 - DNA, 22 bp, unidentified
  source 1..22: mol_type = other DNA; note = PAI-1 (Primer F)
cctcttccacaagtctgatggc

SEQ ID NO: 59 - DNA, 23 bp, unidentified
  source 1..23: mol_type = other DNA; note = PAI-1 (Primer R)
gcagttccacaacgtcatactcg